European Patent Application EP 4 534 697 A1, published April 9, 2025. Title: Method for Detection of Lung Cancer. Applicant: GENOMICTREE, INC. The sequence listing filed with the application follows.

SEQUENCE LISTING (9 sequences)

SEQ ID NO: 1 - DNA, 19 bp, synthetic construct
  misc_feature 1..19: note = Primer
  source 1..19: mol_type = other DNA
cggtacgtataggtatcgc

SEQ ID NO: 2 - DNA, 29 bp, synthetic construct
  misc_feature 1..29: note = Primer
  source 1..29: mol_type = other DNA
ccaaaaccaaattctccgaaacgctcgcg

SEQ ID NO: 3 - DNA, 26 bp, synthetic construct
  misc_feature 1..26: note = Probe
  source 1..26: mol_type = other DNA
cgtattcgcgtgatggttttggatgc

SEQ ID NO: 4 - DNA, 21 bp, synthetic construct
  misc_feature 1..21: note = Primer
  source 1..21: mol_type = other DNA
gagagattgcgcggagtttac

SEQ ID NO: 5 - DNA, 31 bp, synthetic construct
  misc_feature 1..31: note = Primer
  source 1..31: mol_type = other DNA
cgaaaacgaaaaaaccctacgaacacgactc

SEQ ID NO: 6 - DNA, 30 bp, synthetic construct
  misc_feature 1..30: note = Probe
  source 1..30: mol_type = other DNA
tttttgggaaggcgcggagttcggggaagt

SEQ ID NO: 7 - DNA, 26 bp, synthetic construct
  misc_feature 1..26: note = Primer
  source 1..26: mol_type = other DNA
taggagtattagtaatgttaggagta

SEQ ID NO: 8 - DNA, 22 bp, synthetic construct
  misc_feature 1..22: note = Primer
  source 1..22: mol_type = other DNA
ctaccccaaaaaaacccaatcc

SEQ ID NO: 9 - DNA, 27 bp, synthetic construct
  misc_feature 1..27: note = Probe
  source 1..27: mol_type = other DNA
agaagaagggaggggtgttaggagagg